European Patent Specification EP 3 653 732 B1, published May 24, 2023. Title: GENETIC TEST FOR LIVER COPPER ACCUMULATION IN DOGS. Applicant: Mars, Incorporated. The sequence listing filed with the application follows.

SEQUENCE LISTING (238 sequences)

SEQ ID NO: 1 - DNA, 121 bp, Canis familiaris
ctcagaactagataggctaataagtgataggccttgtgttttcctagagtgtgctttaaargtttcttaagctaaaaaattacattcgtgagaaaattgaaataaaaggaaaacagtcatg

SEQ ID NO: 2 - DNA, 121 bp, Canis familiaris
tctcagatacttgatagccagcatttccccccattttcttccaagagcacgaaagcatagraatgatattacatctcgtatggtgaatgtgacacagccgtcagttgcgttagctctgctt

SEQ ID NO: 3 - DNA, 121 bp, Canis familiaris
tattaccctgctctccagccactcctttaccttccattagcccacacctgctctacacacyattgctcatggaagccttgccacgtccagtcgccactctgaaatgccagcatccctccca

SEQ ID NO: 4 - DNA, 121 bp, Canis familiaris
gacctgacagattatgtagactttgttttcaaagggagcacctgctggatatacaacatgrcactaaattgtgctccacatccttggcagaggtggggggcggggcacaaaggaagaaacc

SEQ ID NO: 5 - DNA, 121 bp, Canis familiaris
gggcccagcaagtggcagaactgggaagaccccctcttcttccgcctggagcagtggtgtrgcagcacaccacaggagtctgaaagggtggggagtccaaacgggaacatatacctgagat

SEQ ID NO: 6 - DNA, 121 bp, Canis familiaris
ggcaacagggacaggctgctgggccacacactcacccacactaggagacaagatcctccayatcctgggtctctatcagtcaatcacctagaccagtgggccagaggacagggtccagctg

SEQ ID NO: 7 - DNA, 121 bp, Canis familiaris
gttgagagagatcatacagattcatgtggcaggtgcacactttttctacctcttacaacgyattctctctggccattccttctcctgggtcccaaagtcggagagcttagcgggagcctag

SEQ ID NO: 8 - DNA, 121 bp, Canis familiaris
ataagttcacattttggtgtttcaagtggacatgaatggaggggagggccctgttcaatcyactaaagtgttttttcatcttgtttttgtggaaatcaaatcaagaagcagagttttatgt

SEQ ID NO: 9 - DNA, 121 bp, Canis familiaris
actctcccgatgtgggcaccatatggtggaccactttctgtgtgagatgcctgctcttatygccatgtcctgtgaagacaccatgctggtggaagcatttgcctttgccctgggtgttgcc

SEQ ID NO: 10 - DNA, 121 bp, Canis familiaris
aatctaagtagactgagtggtcaccttcagcgctcagacctgagcatacaaagcatggaargttactgtgattcagctgatgtaatggaatgaaataaatataagagtttggtaacctaat

SEQ ID NO: 11 - DNA, 121 bp, Canis familiaris
tggagagtgctggcaggcaggggcaggcaaacaacaatagcaaagatctcttccacgcttytacttcctcaaaagtccaagccctcttaagatcgcattttcttagtgaccttcactctaa

SEQ ID NO: 12 - DNA, 121 bp, Canis familiaris
ttctttgctaggccaagggcagagaatgcatgcccccccttacctcccagggcccaagagscatcctgagctgagtctatggctcctggtggggggcggctgtgggttgggggggcacaga

SEQ ID NO: 13 - DNA, 121 bp, Canis familiaris
ggtgtcaccaatgccagcgagcaccagctggagggaacaggacacaggtcctccgtcctgygacactcggatctggggctttgcctccaaaacggagaccatgcctgtccatggttctacg

SEQ ID NO: 14 - DNA, 121 bp, Canis familiaris
ctctagaacccttcaggtagactacattcactttctactacaacttcatcaccacaaccawctcccagtaaccccctttttttcttctcctttttttattttttccttctttttgctcgtc

SEQ ID NO: 15 - DNA, 121 bp, Canis familiaris
tcccatgggttgaaggatatctggcagacggctccaactccagtaaagcctcaggcctcarccaggagttccccggggcttcattcccatcccagactttgcccagggctgatttgaaagt

SEQ ID NO: 16 - DNA, 121 bp, Canis familiaris
tcttccttgcagattggatggctgtagcctcacctcacactgttgctgggatctgtccacrcttctgacctccagcaagagcctccgggagctaagcctgggcagcaatgacctgggagat

SEQ ID NO: 17 - DNA, 121 bp, Canis familiaris
tattgctagtaaagccaaactttctattccacaattataaactcatggagatggtaattayagtgcattatttgtcaaattttattattttttcaaatcccaaagaaaatgtgatattcta

SEQ ID NO: 18 - DNA, 121 bp, Canis familiaris
aagaacaaggatacaatctaagtgataatcatccagcatgtacttgtcctgttttcagatkatcagcttaagtcaagaggaatttttagtgcttacaaatatttcaagtgatttttccaga

SEQ ID NO: 19 - DNA, 121 bp, Canis familiaris
tgaaggggtgctactcagggctcttcatttaaccttccaggatgttttcctatgtactcaytcttccttttggttgctccttcttcttgcatttctttatctctttacagaatcatccagg

SEQ ID NO: 20 - DNA, 121 bp, Canis familiaris
acaaccctaaaatttcagtgattcagtacaacaaaggtttattataaccattcagggatcsaagttggtagaaacttcactacaatacctgcttccagtcaacaagacagaaaaagaaaaa

SEQ ID NO: 21 - DNA, 121 bp, Canis familiaris
gcagggttgatatataactagtatgcattaggtagacacctattttgattactcactattktaatatcagcctggtagtaagaaccaaatctattatgtaaagtgcatagagaattgaaag

SEQ ID NO: 22 - DNA, 121 bp, Canis familiaris
ctagctagccacccaactccccacatgcccagagtcatcgtttatcttttcacatcagcaytacattttggcttgcattcaaacattagcccattttttttccttttgttttatttataga

SEQ ID NO: 23 - DNA, 121 bp, Canis familiaris
ttttctctttttccataaatgctctgggcttattttcattatctagtatttctcttctgargctaactcccaaagagttttgtgcatccttatttccatcacaaggtcaatgtacgagtta

SEQ ID NO: 24 - DNA, 121 bp, Canis familiaris
gggcccaagggctgaggatctctgtaccttctgcttcttggcagcccaggctgggtagcakttcttggaagaggatttcccatgagttgttaacagaagggcgggcttccaggcgctgctt

SEQ ID NO: 25 - DNA, 121 bp, Canis familiaris
catctttgcttggggcctggggtttttattgaggattgtgatctggtgtatgtgtctcctyaggcatccagaaaccattcagaacaagaacaagcgtccaggtatcctctgtaagtcactt

SEQ ID NO: 26 - DNA, 121 bp, Canis familiaris
acaaaccctcagacccagatacacagtatcatgtggacacagacatgtaacaccaaaatgmccaacatcatgtgactacaggccctaagcaactaggtgtaacatcacttgggtatgggcc

SEQ ID NO: 27 - DNA, 121 bp, Canis familiaris
aatgcagtaatacatgtagctaaacctaaccatcagagtctgttctatccttctacaaaartagggttggagctgagcacataggtagcatacatctagcaaaagtttttgccttcagatt

SEQ ID NO: 28 - DNA, 121 bp, Canis familiaris
ttgtggggtcaggtgagttatggacccctccctactcttctgctatcttgccccctacagkggttgctattttgatgtaatcacaaaacgacctggcaataaaacctttttctaattaggg

SEQ ID NO: 29 - DNA, 121 bp, Canis familiaris
gatgcaagctgggacagaataaggtactgggctgtgtcaagccccagtaagagaggagcaytgtagggtagttaggatggacttaatggagatgagtcctagggagccacactcagagtta

SEQ ID NO: 30 - DNA, 121 bp, Canis familiaris
taaacacccccaatcactaccatcctcacacctaaggatacacaatgtgtctactttatgrtatgtctttactattcgttgcttatgaaattttattcattawctaaaacagggaaaaaag

SEQ ID NO: 31 - DNA, 121 bp, Canis familiaris
tatagytggscaattaaatctcctattcttttgtctcaaaggatatttgaaattacatagytcttttctcatataaaacctaccatacaatcattagatgatccttcttagttaatttttt

SEQ ID NO: 32 - DNA, 121 bp, Canis familiaris
gatgctgtgggccagtccagaacccacctgagagaaacaaacaggcctctttgccagcagrgcagcgtcagtgtcacccctgtgacatgtcagaacctccctgaaagttcatctaacctct

SEQ ID NO: 33 - DNA, 121 bp, Canis familiaris
ggctcagaagaaaaatcagcccagttcacatccaatgtttccacacatctaatcgtcttgrgttcagaggtagatgtggtatcacttayatggacacatataacagctggcccccacctct

SEQ ID NO: 34 - DNA, 121 bp, Canis familiaris
gtttcagttaattatagtccttactggatccgattgctgtggcgctaaaatgaaagaaggyagggtacctgggtggctcaggggttgagaatctgcttttgactcaggtcatgatcccagg

SEQ ID NO: 35 - DNA, 121 bp, Canis familiaris
cagagtagcattattttctgctgtatgaggacacttttgttatatccacagtggacagaaractgggttttagaacatgctcaattgaaacaagactgagggctcacaaattcctgctcca

SEQ ID NO: 36 - DNA, 121 bp, Canis familiaris
ttacttattcatctgagaccaaggccactgtggtgaacctacaaagccttacaaagcaggrccagaagggcacataaatcacttgactaacatttggtcaaaatagctcttgggctctttt

SEQ ID NO: 37 - DNA, 121 bp, Canis familiaris
ataaaaataaaagagctattaataagaactcataaaatctacataaatatagtaacaggtyaatattcccagcatatttttacaaatcatctataaagagcatgagagcatatagggatta

SEQ ID NO: 38 - DNA, 121 bp, Canis familiaris
gcaacaacctggtttgtgtgtgggaagctaatgcctccccaaatgcagcaaactctcctcytgattttagaaaagcagtttagttacaggcaaatgcatacatgcatgataaatactactc

SEQ ID NO: 39 - DNA, 121 bp, Canis familiaris
gattttataaaacatgatgaccttggcatttatatagtagatattactactctgaaattcsaggaagtatgatcataaactcacacttaatctggtagaagtatggacaatgtatcaaagg

SEQ ID NO: 40 - DNA, 121 bp, Canis familiaris
cttggttgagttaaaacatttgcccatgcaatttaatgcatgtccctgtggggttggaacygacgtacacccgagccaacagcctttcatggcagacgccatcaggcaggtgacccccacc

SEQ ID NO: 41 - DNA, 121 bp, Canis familiaris
ccttccacacgctcaggttggcacggagggggtgtccttgcctgaggggtcctggcacagycatcagggcacacagctgataacccaagggagcagtaggcaagacctcatgggcgccggg

SEQ ID NO: 42 - DNA, 121 bp, Canis familiaris
attctctttgctgtctcctgtatacagagataaaagcaagagttttccccttcaggtttcygaaacccagcttcctttagattttaaggggtattctgtgtacccatttcccaccttctgc

SEQ ID NO: 43 - DNA, 121 bp, Canis familiaris
gcgggttgggacccccccttctgctgctcccacttcagagttgtggcgtcactaagatgasacctcatgtcgggaacctgagagtccctcgggagttgtgcagggactgtagccgacctat

SEQ ID NO: 44 - DNA, 121 bp, Canis familiaris
acatatgcacagtgaatcgtggattgttgtgtttgatttcttacatgatacaataaaaggraagtagttgaagcaaaactttagtttaaaggaaacaatttctctatcataatgttcagtg

SEQ ID NO: 45 - DNA, 121 bp, Canis familiaris
cccacagaccccaggtgctgaccacagcagccacttgggcccccaatgcaggagacacctygggaatgaaggggacaaggccagctcaggcacatcgtcagtgcacctgatgggaaggccg

SEQ ID NO: 46 - DNA, 121 bp, Canis familiaris
atctgatcctagccaatggaaagcaatttgagataggaatcatatcttgttttggtttatrtgctttctttggagttttgcacatcatagataactgtaaatttgtagaataaatgtttga

SEQ ID NO: 47 - DNA, 121 bp, Canis familiaris
gtcaatgccattaacctggcgaagctgctcgagcatccactgcgatctccgcacgaacgaygtggagccttcaaactgtttgaccttcgtgatggatgcttgtgtgggtttcttgtttgtc

SEQ ID NO: 48 - DNA, 121 bp, Canis familiaris
actggttaataagacttcacagattttatccatcatgttgattatctgtatatgtattttytaccacttaggataaagttctgttatctgtaattgattccaaccagcatgtttgctccaa

SEQ ID NO: 49 - DNA, 121 bp, Canis familiaris
cttcttctttcccattggattctttcatcaatcgtaggtagttcttaatgaagatctgtgrtaaagccattcatctattcattcaacaaatggcatcacagaaaagaaaaataacctttat

SEQ ID NO: 50 - DNA, 121 bp, Canis familiaris
gggacacatttctggacagacctctgatcacactcacaggacagcaagaggaagctctggrtacaagtacagggaaaaaagaaagaaatggtcacagggaagctgccgcaggaaaaaggta

SEQ ID NO: 51 - DNA, 121 bp, Canis familiaris
gggcagatcctcagtgagtattggctcatgttctccgagggaagtagagtcccagaagaargatgctaaggtgccaagattcctgagcctgtgtgtggtacagtcacagcagtactcctga

SEQ ID NO: 52 - DNA, 121 bp, Canis familiaris
tcatctccatttgtaatagaaaccacatatatagagagattggattattaaccactaaaaygtagccactcaaggggagggggggaatgcatttggtttatttcccatgtcaaaacagaat

SEQ ID NO: 53 - DNA, 121 bp, Canis familiaris
aacactgctaataaatatttataatggtttgaggaaaatatcaggtgtgagatgtcttcayatcatataatatatcataatatcctctaaaaaagctctaagcataggtctatggaactca

SEQ ID NO: 54 - DNA, 121 bp, Canis familiaris
aagcaatccaggagtctttctccgggtagcaggctcgctttacaggttaaggctggatgaraaggaagaacctgagcttcaaattatcatctgagtagagctgatacccatggttacatta

SEQ ID NO: 55 - DNA, 121 bp, Canis familiaris
gattttattctttactttgattttttttaagttttactatgatattcaatatgattgtggytcatgagattcctctttttagctgtatcattaactacagagcgttctcaaatatttttct

SEQ ID NO: 56 - DNA, 121 bp, Canis familiaris
gtggccggagggggtgggccctactgtggcccagcttcacgtcccactggccaaacatcargatgcagacacccaggtcccttgtgctgcctgctgaggctaggagcagcgactggaaatg

SEQ ID NO: 57 - DNA, 121 bp, Canis familiaris
gatgggagacctcatacacatgcaaagatcactattaaagactctcgagcaaagatcgaayggactgtggcaagctgccgcgcatgccaatcaacaaatgcctccgaccatggatctaacc

SEQ ID NO: 58 - DNA, 121 bp, Canis familiaris
caacaaggtttttaaggttcttttcactaccttcttctttttgtacttgcttaggacaccygtatgtcttcacaatatcacctgaaagtcctttaggagatatactcaaaaaataaataaa

SEQ ID NO: 59 - DNA, 121 bp, Canis familiaris
caacctgagctgaaggcagacactcaactgttgagctacccaggtgtaccaaacacatctrctcttaaccaagcttattctttgctatatttggcaaattgtggcatgtctacagtactca

SEQ ID NO: 60 - DNA, 121 bp, Canis familiaris
attccccatgtttgaggaaatcacaggagccactaggaaatcaaccatttcccaaccaacytgatgatttcctgatccaaaggttctcccaggacaaatatgaggtagcctttcacactct

SEQ ID NO: 61 - DNA, 121 bp, Canis familiaris
cagtcttgtaggagagtagattgactcacagaactggcaagattgggaatctgagcattgycacttgagtcttaaaacgtttacgattttatttctagtatttcaataagaaacacattct

SEQ ID NO: 62 - DNA, 121 bp, Canis familiaris
gaatacattgccagaataatttcaagttctcaaatctcaactaataagattttcgttaaakaaggcattcaatcatcacttactgacaacccacaaaattaggcactgatgaaaaattagc

SEQ ID NO: 63 - DNA, 121 bp, Canis familiaris
aagttaagatattcaagaaagagaagagagtgactgagctaaaaagaaaatcagatctctyccaggctttaaaataatctccacaatactgggcaatccatgtagtctccccagttccatt

SEQ ID NO: 64 - DNA, 121 bp, Canis familiaris
ctcaaaaggaaaagcctgtggaaaggcaaagaggtatgtgaaagaggtaagttcaaaatgstgacatgaccagtgtacatagattacagggtacttggaggagcagtgagaaaggagtcca

SEQ ID NO: 65 - DNA, 121 bp, Canis familiaris
ttctatgaaatagctaccattctggttggtatcttctgttgatttagatgatgaaggaagyataagaagtaaggcttatgagtttataaagctttagttaaagctttgattgtgacaaagc

SEQ ID NO: 66 - DNA, 121 bp, Canis familiaris
agaggagaaaacacagctaaaaacttttttacagactggacaaaggtgcttacacttttcrtattgggcagaatgaggggatgaaaacaccagtggtctttttgaagccacacaaattcag

SEQ ID NO: 67 - DNA, 121 bp, Canis familiaris
aggatgaatatttattaacagtaaatatacatttttattgttctatatactctaaagacarttgtagacagtaagatatatcaattttagaaacagaaataatgttaattgtataatatgg

SEQ ID NO: 68 - DNA, 121 bp, Canis familiaris
cagggattcctaaagggtgacatggtatggtctaacacttcctcactgtccttttcccagmtgatataagaggaggaccagagagacacataaactgtctgagtctttagcattgtgataa

SEQ ID NO: 69 - DNA, 121 bp, Canis familiaris
acactaatgggtagagaatacacgtccatcagtcatcaatgtaatctactaacagcctcasagtctggcagttttcagtgaaaagaggagtcatctccatttattcgatcaatcagttgac

SEQ ID NO: 70 - DNA, 121 bp, Canis familiaris; identical to SEQ ID NO: 3

SEQ ID NO: 71 - DNA, 121 bp, Canis familiaris; identical to SEQ ID NO: 2

SEQ ID NO: 72 - DNA, 121 bp, Canis familiaris
acaggaaggagaactgagcatcaagagagttcagaacatgatcattgggtcagtttgtggstgcattaacttttccccaaaacagaaagcaacagagacttctgtaggtcagtcaacagtg

SEQ ID NO: 73 - DNA, 121 bp, Canis familiaris
ttaccattactataacccaagttatagtatactataaccaagtccttaattgacttgatgyttgtgcagctgattttaaatctatttagaataatagtttacttgtgacaattcatattaa

SEQ ID NO: 74 - DNA, 121 bp, Canis familiaris
ttggtcgactgactgattggttttactgtggaggaaagaaaagggaattttcccaaagagracagagagaaaacatggaattgagcaaagggagaatagagagacagggcagccactgaag

SEQ ID NO: 75 - DNA, 121 bp, Canis familiaris
tgccttatcctccagctcctccctcaccatcttggaaactagctcaaatgtcactggtacktgtctttcttttgatctttctgaaagacaaacatgatcccatcacctctgcctttagaac

SEQ ID NO: 76 - DNA, 121 bp, Canis familiaris
actcctaagtaaaagttaaattaacagatttgccatcaagtaccttgcccatttttcctayagatcgactttttactggatgatccccttgataataatcttgatctatgttttaattcca

SEQ ID NO: 77 - DNA, 121 bp, Canis familiaris
ctggtgggcttgtcaggggcaggatgttgtgtggtgagcacagaattaaaactaggagctygaagcgcctggggggctcagttggttgacggactgccttcatctcaggtcatgatccctg

SEQ ID NO: 78 - DNA, 121 bp, Canis familiaris
catacagcgaagagataaaaacacaggatgctgggctcacgaccatgaccggaaaaggacrgcgaggaaaagcaagtatgagcagcccaaagtcctttttccagcactggccataggagga

SEQ ID NO: 79 - DNA, 121 bp, Canis familiaris
cagagatgaggaatcagactcctcgtcctctgcttctctacaatggctcatgttctccttycccctcagctgttgcattaacagaggtcaacccattcttctaaatttaaatctcccagaa

SEQ ID NO: 80 - DNA, 121 bp, Canis familiaris
aatcaaacaagtgctagaacatagaacaagtggctcatcttttccccaaatgtctggatargaaaaaaaaaatctaaacaaatgctagatgttaagtatctgaaatgatcagcccatgaaa

SEQ ID NO: 81 - DNA, 121 bp, Canis familiaris
tccataccagtccttgttgtctaccccgaacttcacctctctaggcacagacagctctaamtttcactcataggtatcttatgctgacctggcctgcctcctgttttgttttgttttgttt

SEQ ID NO: 82 - DNA, 121 bp, Canis familiaris
caaaaaattccctgagcccagcatcaaggtacctggtttggagtgggtgggtcctcagaamgaatgggtgtggtgtacatttagcaagttatgtagcatgtgtctgtgtagtctcacctct

SEQ ID NO: 83 - DNA, 121 bp, Canis familiaris; identical to SEQ ID NO: 5

SEQ ID NO: 84 - DNA, 121 bp, Canis familiaris
atataatataacttatttaaaatatttgaagatatttctatagttatgctctaccatttgytattataagatttccaacagcttacttcttgtatgaaattaatttaccagcccctcacct

SEQ ID NO: 85 - DNA, 121 bp, Canis familiaris
ccctattctataaacattccctctctggccatcctgtcaagtgggccctgacagtgtgccscagaagctccctagcctttgcccattccagctatggctagcctgccaccagccatacaca

SEQ ID NO: 86 - DNA, 121 bp, Canis familiaris
cactgtgaggtctgaatggagacattcatgatagactccaggattttcccagctattaagycatgggccataaactggaacacttggaaacagtccataggttcatattaaagaatatgtt

SEQ ID NO: 87 - DNA, 121 bp, Canis familiaris
gcaaaaggaacatgagttctgatcttctgtaaaggaggctaatttactaatggtcataacygtggcctgagggtcaagtttctaattaaacgtgcatcttggggyggactagaatactttc

SEQ ID NO: 88 - DNA, 121 bp, Canis familiaris
caaggsccaggtaccctgaaggagtccgcttcacccaggcatgatgtgtttgacagtcttygtaattgatacagccattggcatcctcttgcggccaayatcagctccacttcaacctcgg

SEQ ID NO: 89 - DNA, 121 bp, Canis familiaris
tgcaatgggttttgaaattagaggacatcacagcagagtagaatggtttggaacaggggartatgattaggattaatgagatgaaagaaaattctggctagagggctagaagagccatgga

SEQ ID NO: 90 - DNA, 121 bp, Canis familiaris; identical to SEQ ID NO: 1

SEQ ID NO: 91 - DNA, 121 bp, Canis familiaris
gatactttgggctctgggtgggagccagcagtggtggggcagggcaggagtccagcaaggygtctgggcatacatgtctgagagtaggaaaaccacaccattgcaccttgcctttgacttc

SEQ ID NO: 92 - DNA, 121 bp, Canis familiaris
tcaaggatcagaaaaataaaagcaaagaaagaggcaaagaaagaagaaatgaaatacctartggcagaagtaggcagagaaataaaggctaaaagaaaatggcagaggattgtttgaaagg

SEQ ID NO: 93 - DNA, 121 bp, Canis familiaris
tatgttatactattttagtatcttaataaatatgattagccaaaatagttttatcatcctsaaaagtgcagcatatattattttctattaaattcagaataggtataaactagaaagcatt

SEQ ID NO: 94 - DNA, 121 bp, Canis familiaris
acagcagttctgaggatggactcgcagaggctcctgacaagcagaatgaccaggccgagcrgaaaggtcagtgctgccagtctagccagaagtgggggagagaggatgtaggagcagtact

SEQ ID NO: 95 - DNA, 121 bp, Canis familiaris
actgtactcaaaaaagttctgtttgcctaaatgggatcagcctctaatggatgccagtgaygggaggctgttcatcatcccttcgggataattcagagcctaggcagaggcccagcgttca

SEQ ID NO: 96 - DNA, 121 bp, Canis familiaris
tacaggccccaggaaggagccaccagatgcccaggactgggcccaggaatgatggaggctrtacagctggctgcctgcactggctgccgcccctgtcatccagtgtcacagagcagcacct

SEQ ID NO: 97 - DNA, 121 bp, Canis familiaris
agacattgccaagaagtatccacaatgaacagtttgaaggggatccagaaaagcacagggyctacttccgctggatgagcagcagtgagaaccacagtcaggtaggtcttaaagcaaagtt

SEQ ID NO: 98 - DNA, 121 bp, Canis familiaris
gctttgaaaaccaacaggaaatacatccaggaaagctatacaactgtggtgaaaggaaagraaaatctgctcttaaaaggttgtgtgcagactcacttgccccagaaaccagtgcgaaaac

SEQ ID NO: 99 - DNA, 121 bp, Canis familiaris
gagatgtgtaaaatttaatagaaatgaaacttgccaaaacagacctctgtactcgtcagcrttctaagtccatctttctgtagcatgtaagtagaataatgttctattaatttcctctatg

SEQ ID NO: 100 - DNA, 121 bp, Canis familiaris
gttctttctattctatcacacataccacccccctgcccacagtacccctttctgccatgtytcagactcctacacaagaggttctctctcctggcttccagttagacaggcaggtaaagct

SEQ ID NO: 101 - DNA, 121 bp, Canis familiaris
taaaaaaatacaacagtagcattagaagacatgctaagcggctgtattagagaaggttagygctggcctgaagtttagaaaccttcccttctctttttttttttccttcccttctctttaa

SEQ ID NO: 102 - DNA, 121 bp, Canis familiaris
tcaagagtactagagcatctataatcaatggtaaattggggaactagtgaaacaagtttayaggacaaataacataaataaggatttttttttaaatttggaaaattgtggaataatgata

SEQ ID NO: 103 - DNA, 121 bp, Canis familiaris
agaattcaattttggggagccaggaaaccagattagttttccaaagggaagtgccatttgyatctatcccggtggggctgccaagaattccctggggtgggagacggcgcttctgtggatt

SEQ ID NO: 104 - DNA, 121 bp, Canis familiaris
caccagagagccccgcaagatcatactgcacaagggctccactggcctgggcttcaacatygtaggaggagaggatggagaaggcatttttgtttccttcatcctggcaggaggcccagct

SEQ ID NO: 105 - DNA, 121 bp, Canis familiaris
tggtgatgatttatcccccatgttcaagatttatcctccctgtctcaagaaatcatgtcaytacaggcatccttaaagtcacaagactgggaagtaaatactgatgaggtccaagacctgg

SEQ ID NO: 106 - DNA, 121 bp, Canis familiaris
agcatagtgtacccacatataaggtcacatctgaggccagggagtcggggtcttgaagatkatgactgatcatgtgcttgaggatgatgatgatcatgtgcttttcctggctgtgcagttg

SEQ ID NO: 107 - DNA, 121 bp, Canis familiaris
gtgtgtgtgtgtgtgtgtgtgtgtttaattctttgtgagaagcccctcattttgacctaartttggtagaggccccaggggatctgagaggagaacaaaaggataaaccatttgctgttca

SEQ ID NO: 108 - DNA, 121 bp, Canis familiaris
ccaactttcactagcatcacagcccctatcaatctctgttcttttttctgtcagtaccatrtttgctcctactacatcyaatctgtgagctcacaggatgaggaccaacagctgccctgag

SEQ ID NO: 109 - DNA, 121 bp, Canis familiaris
tgtcttacctctctctattcccttgtccatagtagtattaaatatatcttcctgaacacaratctgatccagtctctttttgtaattaaaagcctttgctagctttggtgatcacctccag

SEQ ID NO: 110 - DNA, 121 bp, Canis familiaris; identical to SEQ ID NO: 4

SEQ ID NO: 111 - DNA, 121 bp, Canis familiaris
cagaggaaaaggagaaggtcccacttaggggactggagaggagtgggggaacatcaccagmgccttcctgagccaggccccctgtggggagaagctctccccaggactgggtgcctttgaa

SEQ ID NO: 112 - DNA, 121 bp, Canis familiaris
tcctccctctccccatccccattctcatgcaagtgtgctctctctctaaaacacccccccmcacacacacacacagacacaaccaaatttgggtctcaatgtcttgaccaaggaaaaggca

SEQ ID NO: 113 - DNA, 121 bp, Canis familiaris
gagaagaaggaggagaaagaggaaaagtatatttgatggaatgaaaaacaagagttcaatytcactctggtctggggtgaccactattagtccttcaacatcttccttgaaggaattttaa

SEQ ID NO: 114 - DNA, 121 bp, Canis familiaris
ctggaattctgtcagatcaacattcagagctccatcaaatctgagggaagcagtgatagargatacaatttgacctttcagtctattcaggttcatgtaggttaggcattcaatatcaaag

SEQ ID NO: 115 - DNA, 121 bp, Canis familiaris
ccacatgtggttacaccactgtgttatccttccacctgtcccatcaacccacccgcacatrtcacagtgcctctgtcctcaaagaacactgtatccaacacctccacatcctctcagcatg

SEQ ID NO: 116 - DNA, 121 bp, Canis familiaris
attcctatggtgggcgctgcacatttcctcccaggggaagggcaagggtcctgcatttctrtgctttccagggcctccgcaccaagagcaattgctaggtcacgcatgcccctgcacttcc

SEQ ID NO: 117 - DNA, 121 bp, Canis familiaris
catgtcatcactaactaatttattaacaagagttttattctttgaaaaacaaaatcactcrcattactcagttgcttattccttgattcatatacaaatgactgataacatgagataaaaa

SEQ ID NO: 118 - DNA, 121 bp, Canis familiaris
gatgatttagttgtttgaatgatctggcatataaatcttccaaatctgtgtccattggatygcttacagtttaatctttttatttcttcccagaatcacattttttcattatttatctttg

SEQ ID NO: 119 - DNA, 121 bp, Canis familiaris
agttaaattctgtgaataactagaatccgttatactttttctgaaatgaagtctgtaggcwtttcaacagcaaaaggaattctgwttttyaaaactatacataatgcttcttaaaagccct

SEQ ID NO: 120 - DNA, 121 bp, Canis familiaris
aatgccaactttaaaaacgcattcaaggttttcctctgtaaatgcattcctcattttggaygtgatgtaaaatcttattcagtgttttgtttttttttccccccacaggtctcaacaatta

SEQ ID NO: 121 - DNA, 121 bp, Canis familiaris
ggtgggaccggccatcagcaggcgggccagcgccccacagatgttgtcacggacccgatcrtggcgctcccgtgccaggaggggcaacagaagccccagcagcttggggaagtatctggtt

SEQ ID NO: 122 - DNA, 121 bp, Canis familiaris
aggggacttgtgctaatcactgggcaaattttatgaacttctgaattttaaagcaaaagaraaggtgaaagaatggaaagaaggtgtgagtgtttgaggaaaacttcttctttggggttga

SEQ ID NO: 123 - DNA, 121 bp, Canis familiaris
tacacaagcaaggcagtatgccctgtctccttcccttgggccacctgcacttagacatggyaggttccagtgatgtgtctagtctctagcaagcagggcttgcttctgctctatccatcca

SEQ ID NO: 124 - DNA, 121 bp, Canis familiaris
ctgtccttggtctggacctgctgtgaagaccaagtgcttcctgagatctctctgagtctartttccagagcagtgagtgagaaatgaaatgagccgaggattgccctccctcctatggact

SEQ ID NO: 125 - DNA, 121 bp, Canis familiaris
taagccatcagcatgggctcctaggggtctgttcaactcccttgtggtgtcttactgctcragcaaaggaacagtctggtacagtgggagcaagagctgaggttggagagtggggacacag

SEQ ID NO: 126 - DNA, 121 bp, Canis familiaris
gaggaggtggaagtgattaagtttaaaatttctggggtggtttctggcgacatgaagctgmgagctagaatgcctttcaatctcataatttctttaatttggtgattataccagagccaca

SEQ ID NO: 127 - DNA, 121 bp, Canis familiaris
cctgacaaacactacctctgctcttcaaaagcaataagcatttattctgtgacacatttaratacaaagtcaattacaatagagtataagtacaatactagggaaagtacaaagtcatayg

SEQ ID NO: 128 - DNA, 121 bp, Canis familiaris
gcatgatgaaatcagaaaaagtatgtaagtttctagaagaagctagatatatggtaacttwggtcaaatagaaccatgtagtgaaaagaatatgagttttcaagttcaataaaaaacaaaa

SEQ ID NO: 129 - DNA, 121 bp, Canis familiaris
atgcataagtttccaaaagagttcaggattccaaaataaaagcttcactaaaagattcatmgcaaaagagtaatgaacaattaaagtcataggatatctaaaatgaaaaactgttagactg

SEQ ID NO: 130 - DNA, 121 bp, Canis familiaris
agatggcttagttgtttctctttcctcctgaagtccacagcttagttacttggactctccraaataggatcgttggacatttgaggaaagctctagcatgaaagccatagactaaaaaaca

SEQ ID NO: 131 - DNA, 283 bp, Canis familiaris
ctctcattttgtgtattgatttgaggactctgtcctttttgttctcttaggtgttttgtaaccatttttgtggttcttgccacaaaaggccttatgaagtcctgcatatgagtgatgtgcaggacaactttgactttctgacagccagtttttgtgttttgttmccttagttcccaagttcctatcttgtttacctcatgatcacattttaatatcaatgaaatttgtaggaaaacagcagaaggaaagatataaggttactattctctatggaccttggttg

SEQ ID NO: 132 - DNA, 223 bp, Canis familiaris
ttgcagattatatgataaatatagttgtagcttcaaaaatgactataacgaacagaaaaaaattaacttatcaaaaacttttcaaatttccccatayacttaactaggtaggccacagagtatgatagtatgcaagttattaaaatctgttagcaaggcataacacatatatttctacttaatgaggtttctataatcaaggcttgtcaagtccattatgttc

SEQ ID NO: 133 - DNA, 157 bp, Canis familiaris
tcagactgaatctaaagccacatatatttcctcagcagctgataacattagaaatcagaaagccactatyttagctggcaccgcaaatgtaaaagtaggctctaggacgccagtggaggcttcccatcctattgaaaatgcatctgttcctaggcca

SEQ ID NO: 134 - DNA, 179 bp, Canis familiaris
tcttgtgcttgttctttatcaccattcattcagtacatccaaattttgaaatccttagagctctatagcctctatgtaggagaatgaratttcatcaaaaggaaatattttgagaatttaagtgatttttttatgatattttagctatagcagtcaccttgagccaaaagacattctac

SEQ ID NO: 135 - DNA, 191 bp, Canis familiaris
aaaaatatactctctttcttacagaaacctctaataattcagattctggccatgaagttcaggaggattcttcaaaggaaaatgtatcatcaagtgctgcctcyactgaccacaacccaacacctactcatgatggcaaatcmcmtraactgtytawtytcsgattggrrawtmaaykgttraggaatgaa

SEQ ID NO: 136 - DNA, 244 bp, Canis familiaris
tttgcccaagaaaaatgaagacctatgaccatggaaagacttgatacataatgctggagtactagtagtcagacccacccaagtcttttcacgtgttcattcagtatagatgcggcacacgttggctgagtccctccgktgtgtcaggaactgttttaggtattggggatgaagtagggaacactgatttagsttctgtttattcatgtctcactttgtaggaattycmhtamatagaaraada

SEQ ID NO: 137 - DNA, 251 bp, Canis familiaris
tctcagtactcacaggtacttacaaatacaacactaagaggtttcacaaaacagtactcttacatagcacatgctgtactctctgttccattctattttattactattttaaaatatggattgtgatytgccaakttgattctctggcccattaatagtttgaaaatctcttctgtaggagtataggaattaccacagagttttgagaaattgatgaatgccacgctttacctgtgggaacgtagattcta

SEQ ID NO: 138 - DNA, 191 bp, Canis familiaris
cagatgatgagtctggagctggtgatctgggctggagataatgaacctgggagtcatcagctttggagaaagggtgtctggcctcactcttgctwgcacagaaagaaagtgctcattagtgtcaactctcagcaacacttggtatttgtaaactttaatttttgctgacttcatggagaaataatgttttt

SEQ ID NO: 139 - DNA, 206 bp, Canis familiaris
taatgatacagaaatgaatttggcaggaatgtatggaaaagtccgaaaagctgctagttcaattgaccagtttaggtaagcaagtgcagtactggtgaggaatggkgcatcggctccttctgtgctattttccggtggctccagtcacagccccatcaagcagagctgatacctaaagtgacatttaccctacttcctctctcaat

SEQ ID NO: 140 - DNA, 186 bp, Canis familiaris
catcacttaaaatcatctcagcaagtgttgttgaagatgattttttataaagtatattccaatcttattctatacttcagaagcttggaattctyatttgctttgctggattgaaaaagtctggaagtaattagaatgacttctcatactcccaccttgaattctcctaatatcaaaggctgggag

SEQ ID NO: 141 - DNA, 171 bp, Canis familiaris
  misc_feature (169)..(169): n is a, c, g, or t
atatggagaaatgagctcttatacactttcagtggacatgtaaactgttattgtctttttggagagcatttggcaggatctatcaaagtrcacacatcatttgattgagcaattccacttccagccatattctggacataatttacaagtataaaaagatgcatgtttnga

SEQ ID NO: 142 - DNA, 213 bp, Canis familiaris
aaatattgaaagtgctttatctacactccaatatgtaagcagcatagtagtttctttagagaatagatctgccatagtaaagtacaatgcaagcttagtcaytccagaaaccctgagaaaagcaatagaggccatatcaccaggacaatacagagttagtattgctagtgaagttgagagtacctcaaactctccctccagctcacctcttca

SEQ ID NO: 143 - DNA, 125 bp, Canis familiaris
ttaaaataactacttgcagtgatttctttcccccagtataaaatgtcagttttgtctcaatccacccycttcaccttaaaaagaaaaagaaagtattagttttcagtgtcatttgccttaaaatg

SEQ ID NO: 144 - DNA, 201 bp, Canis familiaris
gagaggtacgaggcccaggcgcagggccgcatgaagcccctgacggcgtcccaggtcagcgtgcacattggcatggatgaccggcggtgggactccccgcrggccacgccctgggaccaggtcagccgtgtcagccaggtgtctctgtcctccctgaagtccgacaagctgtcccgacacagcgccgcggccgacgacggc

SEQ ID NO: 145 - DNA, 201 bp, Canis familiaris
ggtctgcatttggaacacctgcccagtggttgttaaatttaacccctgctaagagaatgagaggacagcacccctggagagacagaatccaggtgcttgcrgttctccatacgtgcactgcagcaggatccccagagttcaagcaccaagttctgcagggagattgcaggtcgcagcagaggtgctgttgtgctcgttctg

SEQ ID NO: 146 - DNA, 201 bp, Canis familiaris
  misc_feature (8)..(8): n is a, c, g, or t
  misc_feature (65)..(65): n is a, c, g, or t
  misc_feature (148)..(148): n is a, c, g, or t
  misc_feature (152)..(152): n is a, c, g, or t
  misc_feature (181)..(181): n is a, c, g, or t
cggggctngatctcacgaccctgacatagtgacctgagccaaaaccaagagttggacgctcaatngactgagcctcccgggagccccaaagtcaagagacrctacagatgcgttgggcacaatgacaggggaggaagctgaggtctgntggnggaggttctgcacctcccagcaggacccngcacacagcaggtgcctgct

SEQ ID NO: 147 - DNA, 201 bp, Canis familiaris
ggggagtccggcatggccccctgtcagccctgtcccctcagggtgtcttggccgggttgctccctgacaagctctccctcctctctcttcaggttcagccygaatctgacaccatgcccctagggaagagcagcgagctttggaagcagggagaagacctataggaggccgagggcctggggatgcccagctgtctggggc

SEQ ID NO: 148 - DNA, 201 bp, Canis familiaris
ccttcagagagaacccaggacaattactaaactaccgtgccctggaagatgttttgtgactcctcactccctctgccttgcttattggccattattttttkatccctctctcttctaccattattaatcaaacacaacaaacaaaacacttctaacaaggatattaggtttgtatacattttttttaaaaacagcaactta

SEQ ID NO: 149 - DNA, 201 bp, Canis familiaris
acttcctgattgctactgtctggacactaggttttgcgatttgttctccccttccagtgtttcacagtctggtggaacttcaggaaacatttgactccgcrttgctgagcagcaggtatttatgtgttgagtcgtggccatctgattcgtacagaatcgcttttactatctctttattgctagtccagtatattcttccct

SEQ ID NO: 150 - DNA, 201 bp, Canis familiaris
cagggaacattttcaaagatgtagaaaatcccaagacatgttaacatagggaatgcatgtaaagatgcaatcaaaagcctttgaaatgacaaccacttatrtaagacctagcaatgtgcacttccaaacattaactaaaagttctatctcccccctctgggttccttaaacattacacctctctgcctatcaaagcaccta

SEQ ID NO: 151 - DNA, 201 bp, Canis familiaris
ttcctcataggaaatttggccttctctgatattttggttgtgctgttttgctcaccttttacactgacctctgtcctgctggatcagtggatgtttggcaragtcatgtgtcacattatgccttttcttcaatgtgtgtcagttctggtttcaactttaattctaatatcaattgccattgtcaggtatcatatgatcaag

SEQ ID NO: 152 - DNA, 201 bp, Canis familiaris
atccagaagaagtctgctaggggtaactatcttttcgctctctgtttatgccaacatttcacaaaagcttgtctcccgtgacttaaatagatacacccagmgtgtatgttggggatttttgcaagtatccttaggaggccctacgtcgtaaggcacagtcataagacctcgcgtccctattccctcatctgtaaaatggtg

SEQ ID NO: 153 - DNA, 201 bp, Canis familiaris
caaggtctgtggatgtgcttactccgtcctcaccacaaacaccgatgtctcggacacactcagtgagcccaggttaggaagccaggattgcagggccaagrgtataaggaggtgtcctgggagcctcaaaagaaaaatacaaaagtatgaagactcagaataaattcttacaaatcttgctgtgtcttcccacagatggca

SEQ ID NO: 154 - DNA, 201 bp, Canis familiaris
gaaaggccgtttcctacctcggccccaagtagtgagggcctggaccctgagcccatgatggaccaaagggagcaggtgggtgaggccccagcccttggacrgaatatttcattagctaatgcaaatcatgagttcagggaatcctcacagccccctgagaatacgcagagcactgtgttatgtctcccagggtccctttta

SEQ ID NO: 155 - DNA, 201 bp, Canis familiaris
  misc_feature (56)..(56): n is a, c, g, or t
  misc_feature (100)..(100): n is a, c, g, or t
  misc_feature (130)..(130): n is a, c, g, or t
aaagtatcagcacactgatgcagccagcctagctgaagatggagttgttgaagcanaggtgttcatgatccctccccagtgacctgcgattttttttttnwaatcttattcgcccattttattaaatccncaaattcaaatctgtttgtctcacttgctgagatttcttttgtctttctctttcattcattcttacagttg

SEQ ID NO: 156 - DNA, 201 bp, Canis familiaris
  misc_feature (101)..(101): n is cytosine or there is no nucleotide present
aagaaaaagaaaaacccagccatcaagggtgtgcatgtctgtgaaagctccagacaggatgatcgaggttgtttgcaacgacagtctagagaagaaggtgngcgttaagtgcaacactgatgacaccatcggggaccttaagaagctgattgcagcccagactggcacctgttggaacaagaccatcctgaagaagtggta

SEQ ID NO: 157 - DNA, 201 bp, Canis familiaris
gcctagcattattcctgacatgtgttaggtcctcaacaaatagtagctaatatactttctggatttctttctttttggctaagtagaagagctggtgctgycatccttatagtctgtatagtaggatttcttttctttccttttcttttttaaagattttacttatttactcatgagagacacagactgagagagagaggc

SEQ ID NO: 158 - DNA, 201 bp, Canis familiaris
agagagaggagaagcaggctctatgcaggaagcccgatgtgggactcgatcccaggtctccaggatcatgccctgagccaaaggcaagacgctcaaccacwtagccacccaggcgtcccttttaccttagtttttgtcctaaagcttcatataaatggaatcatgtagtatgtatgtgtgtacactctcttttctgacttc

SEQ ID NO: 159 - DNA, 237 bp, Canis familiaris
tgcctctccactactcactcttctcttgaaagattatttcctgcttaaactggcccgtgacttcctgctgccagaaccatggaatggcctcctgagggaggctccctatgctgctcccatyagcagatattgcagcgtcacagtataactcagtggcttgaaatgatggctatttatcattgctcagtaatttgagtggctcgaagaggatagaatttcatttctttctcagataat

SEQ ID NO: 160 - DNA, 237 bp, Canis familiaris
tgtacagctgactccctgagaaaggacatcctgggtcacctttcaagtatttcctggcatggaaaccccatatcttcaaacacaaaaatcagaaaatcacagtccttatctgtttgggccyatttataggagagtctttttattgcctggaattgtatatttttacatttcttagatttctacaaaataatatttgtgccttctttcaagtataatattatttattaaagttgcttt

SEQ ID NO: 161 - DNA, 237 bp, Canis familiaris
attaatacattcttagtgtcttctttaaaaatgcaacttccatgctttataaaataccaacaaatgctttacatctttatgatggtaattttggatcaatactggaggattttaaaaaaayctctgcttcccctgcttgtgtggtctctcacgcgctctcattctcactctgtcaaataaataaacaaaatctttccaaaaagacaaagtccttgtgaaaactgagaaggcctgtga

SEQ ID NO: 162 - DNA, 237 bp, Canis familiaris
atttgtactttcttttcacttctcctgcgtggtgcgtatctctccagtctgtgttctttaggcatacattgctgtatgtgctttaaatagaatcctaccttatatactgcttaataacctrtgaccataagatcaggttccatgtcttcaaagattctcctcatcattttcacgggtataggcatagattacaattgatccattccccactttgcacatttagattgttttcacttt

SEQ ID NO: 163 - DNA, 237 bp, Canis familiaris
tgcaatgactctgtttacaaataaggtcacaatctcaggtaccagagcttagggcttcaacctgtcttgggggagggtgggcaggataccattcagtccataacagcagaagatcccggtygtcctcacagtatggtgggcagtggccagccctccggactttcacctccagggggcaggcggagaagctaaaggggggtctcatggcctcccagctcctccctttgcccctgcaat

SEQ ID NO: 164 - DNA, 237 bp, Canis familiaris
acccacgcccagcatctaagaggccaacccctccctgctgtgggctcctgggcttctcaacccccaaggaggggactgcagtccagcgtgccgacagctgcctccaccccaaagggggccratggctggtgagtggagactgagtgcatgaccgacttttttagccaagactttttcttaattgttagagatggcaaactcaagcaaatgggaaactcatccgctcaagtaaccagc

SEQ ID NO: 165 - DNA, 237 bp, Canis familiaris
gcctcgtgggacagctttctagcactttcccctttttaagagattgactgcaatttctataataacatcacattagctagaaattaatgtcctcattaagacagcaattaggcacattagygcggcaataaaagagaagcttatgaaataattgctggttccgaaatgcctttaatttagtgttttatattgcgccatgttattaattttttccctcggcagaagataataagagaa

SEQ ID NO: 166 - DNA, 237 bp, Canis familiaris
cataaatgccccccccacctctgtgtctgtgcagaaaccaaaagtcttgggcttctatgatccccagtgagtgctaggagcaggaccgcaatcacagcagcacatcctagaaaggacttargagccagatactaccatcctattcactcaggtaatcctcacagtaaaccgcaatggcataaaaaatattacctccagggcccaacggacggactcttgatctcagggttgtgagtt

SEQ ID NO: 167 - DNA, 237 bp, Canis familiaris
atgagatatgtctgctcagccactgtctggggccttgtaattgaagccttataattagcatgaagtcaccagcttggtcctgctgaaagggcacagggtggggtgtgaaaggaggatggcyaagggctcgtccacaggaaacattttctaaacactagagaggaggcagccaaagagctcccttcctcatcgcccatggaccccactgctatgctggcaattccccttttggttaat

SEQ ID NO: 168 - DNA, 237 bp, Canis familiaris
ttcctgtgcagagggacacgtgaaggccctaggtcctcctgggagaaaagatttccctcctaatgatccagggactaggatttcattctgaaatggaatggagaatggcaggtgtggcttkctggggattgagaaccacaggccccaggagattcaggaaaggacagtaatgccctgctgctcaggccccggtggaggaatcatatcctcagctcagcaacaccacccgccccccta

SEQ ID NO: 169 - DNA, 237 bp, Canis familiaris
acatcggctaaacaaaaacaggagaatcccattataagacggttcctgtagtacagatgtgtctgggtgaagcctgggttgtatcgtggccccatgtagagccagcctgggcagagagctrgtctacccactaagcaactgcaagaggcaaagtgcagcattgatgtcacgaggtccagcatcaactaggaccatccccatccatgtgagcaggctcacacgtggaatcgcagtgga

SEQ ID NO: 170 - DNA, 237 bp, Canis familiaris
ccgtgcttcacaggcgagaatctgaatgaccgtgatgccaccacatgtcaccatccccttttccactgggaaaggggtccttgttgccttccagctccagaattgcatcctcacaatttcrgaggcccttcctcctgctaagctctgtgcttttccagaaagtagagcataagacaagggcttatatgcaagtatattttttggaaaatatgatcccagagagcaggagtgagaact

SEQ ID NO: 171 - DNA, 237 bp, Canis familiaris
actccatgaaatggtttattttatcctatgaatcgatgtggagaacaaaggcaaaagaaatatagaaaaatattaaatttccttacaatgtacagcccattgataatattttagacagtgwgagtgatcttgcttatggagctcaactgcctcaatgttaatccttagctaaaggcaaaagacaatcttagtttgacattagcctgaccgccttatgctatccctaacccccgtccc

SEQ ID NO: 172 - DNA, 237 bp, Canis familiaris
aatccaaatactccatgaaatggtttattttatcctatgaatcgatgtggagaacaaaggcaaaagaaatatagaaaaatattaaatttccttacaatgtacagcccattgataatatttkagacagtgtgagtgatcttgcttatggagctcaactgcctcaatgttaatccttagctaaaggcaaaagacaatcttagtttgacattagcctgaccgccttatgctatccctaac

SEQ ID NO: 173 - DNA, 237 bp, Canis familiaris
aggaaaaatatgcttgcttttgaaggaatcaatttgtggtttcttttaatgagttatcaaactattaataagcattaattatttattgtgtaaggcaaagtgcttcttaataggtattctktccttaacttagaacattcacagattcccaatagcctctagtgcagaagaagtctgccgctcttctttcctcctttcactagtctctcctatatctgtgatacctccaatcatagc

SEQ ID NO: 174 - DNA, 237 bp, Canis familiaris
cttccatgttctgtctccctttctgatatttcctactcattccagaaaatattcttaatgaagcctctgatacggtcttgaggatcctcagagaccatatgtcagtctgtcaatgaagcaraaatcaagatgtttggatccctagtagatatgtaatcaaaatgccatgggaatacagagaaggggagtcatttgtatcagttagtgttaaaaattattatcacgctcttgatatta

SEQ ID NO: 175 - DNA, 237 bp, Canis familiaris
gagaatactgaagacgtaatgaagttgagttccacctttataataattccgttttaccctaaaggggaatattcaaaaatgtgacatcgctctaccagaccaccttgcgactgctctaaamgattggcaggggcaagaacttgtgtcactgataggcgggattttttagtcctctctgcaaatcattaagaaaatgttccaacgcaacaaaacaaaatatggtggcgatccctgaac

SEQ ID NO: 176 - DNA, 237 bp, Canis familiaris
acctgataacaccgcctcagtggagaacgagttggcacttcaggacagatttccctgccagagcctattcctgtttgacactttcatttgaagaaacccactcatggtttcttctctccarggtttaaaaccgagatcaagtatatctctttaataatgtcacattccaaagaatgactccgataaggggattgttcaagggcttgggtattcacataagggctatcatgcggggag

SEQ ID NO: 177 - DNA, 236 bp, Canis familiaris
tcctctagatctgacctacatttcaaaaatatatgagtgggctataaccaggaatgtcttctcttgctgccattattcacactgcattttctgaagttgtttttttttttttttttttttycccctcggtgactttaatggccattgagggaactgtagacattgggagtctttatacagccctagtgaaatggcgagtgttatcaatagggtggctgaatggtacggctctgggc

SEQ ID NO: 178 - DNA, 237 bp, Canis familiaris
catctgtgacccttggattcaaaccaagtaggatgcaaacctcagaacttctggcatttcggatgcactgatctctgccagccccttgccctcttctaatgggatagaagctgatgatgtragacaccgcgtgcaccatctgcccaagacgtcccagttgatgccactcatcctggtttgtgcaaaaaattctctatttgccctaattccaccgctcagcaactggaaggacctgag

SEQ ID NO: 179 - DNA, 237 bp, Canis familiaris
tcacaatggcttttttttttttaagatttaacaggaattttgtgatcctttatatgatatgtttcaatgaagccttttgggaaaggttcttaatgtgaaagaattttcacagagaatatcrgaaataaatgtgcaaaagggagtcgttttaggattagagatatgcatggaagagggaaaaagcctacttatattactagaaaataattttcaatttagaagttatactgaactatt

SEQ ID NO: 180 - DNA, 237 bp, Canis familiaris
cccatttttttaggattgataaactgatcatctaacagatattatatacaaaagtcagagaagacacaatagccaaccctgtgtgtaaggaaaatgacagagttggttaaagagaaaagaraaaggaggtacacagagagatgtagaggtcacattaaaaatgaacgttgtccatgtctatgaaagatggaaggtaattctatgcctataaggtatgttataagttaaattaattgt

SEQ ID NO: 181 - DNA, 237 bp, Canis familiaris
aacaaacctaccaaacaggacaaaccagtccggattatataatatgtaaatatgccagggagctggggagcatacttgtgggaggataagctggagcaatggttaaatgagctcaatcctyactatacttgaaggtagtagcctcttcattcacactccatggctagccctttgtaactaaaatatggaaaacacaaccaatgaagaagttacatgtatccctaaaaataccaccta

SEQ ID NO: 182 - DNA, 121 bp, Canis familiaris
cccttggcgttctaaagtccagccccctctcttcgcattctgtgctttctcctgtgtggcrgtctctgtgctttatctgcacataaacacttcacaaatttccgttccagcttagttctct

SEQ ID NO: 183 - DNA, 237 bp, Canis familiaris
ttaagtttagaaaaaacaaattcaagaacaagctttttatatttaacatcgatgaatcagaagatacggggttttttaaattattaaactaaaattattaaactggtcctgtttggtataragttatcttaattatgctaatctggaatcttaaagcatttttaaactaatattttaagaaaccaagttttagatttattccaaccttgggctagaaaaggatgacctttgtgggcc

SEQ ID NO: 184 - DNA, 237 bp, Canis familiaris
tgagccacccaggtgccccaaaacatgattagtcttgaaacaaagtgtatcacaataatgattcaattagatgaataaaatgtagtttttgagaatggtaaacactatgtaagagtaaagytagcctatttgatcagtaaacctatttaagtttagaaaaaacaaattcaagaacaagctttttatatttaacatcgatgaatcagaagatacggggttttttaaattattaaacta

SEQ ID NO: 185 - DNA, 237 bp, Canis familiaris
agatgtcatgctatgatatatttaaataagttacagacatgtataatttccatggtatgttttacattcatataaaaattaactattcataaaatataataaaatgtagtgtttttcttaytgagcttcagtgatcataatttgtatattaacttaatgaccagaaataattaagtaaagctagttaaattcttgggatgttatggattatgttatttggttggctgttcatgataa

SEQ ID NO: 186 - DNA, 120 bp, Canis familiaris
tgttttgaatttaaggtgtttttccaggctgagaagaaacgtgagctcttggaaattatrattaacgtatctaatgcatataccctagagggcaaggaaatttctattcattccctgtat

SEQ ID NO: 187 - DNA, 237 bp, Canis familiaris
cccccaggatctgtcagtaatccctgactgcctgcagaccacatggggagagggatccattcctatgacagagaatttatactggcttgtgagctgaacagatacctcagaagatgttcayctgtgagacagagagacatggtgacaaatacaagtgtcagccaacagcagcaccaagtccaggaatggctgcctgagctggatggaacctcactatccagagccatccataggccg

SEQ ID NO: 188 - DNA, 121 bp, Canis familiaris
agagccaacgctggatctcagggagaatctagaaggccagctgaccagaaaaccaactggrcagacagaagctgggagcagcgcctgtggaggcaggcacgagaggccccggtgcagccgc

SEQ ID NO: 189 - DNA, 237 bp, Canis familiaris
ctgggtggctgttggagagagtgtgttgtgttgttcccagggttagtcctaggaatggtagagcctgtcaagttctccctgaaagtcacgtcactccccacttcagcaggcccagcctgtsttgtatccctgcagcactgcctcaggatccttgctctgcagtgatcagagtcatctgataagcctgtccctgtctaggctgatattaatttcaggttgtcaccctctatgcctctt

SEQ ID NO: 190 - DNA, 237 bp, Canis familiaris
ggccttatgaagacttctctgatctgttgatctgatgtacccagattctgaatccctaattagactcaattaggacactcctggaggtgactactgctttcttagactttgtcactcaaayatctaatacattcgactttgacccatggatttattgagttcctcttgcacacccagttcagtagatgtggtccactattttggtgcatcgactgctctagaatttagcttttggaa

SEQ ID NO: 191 - DNA, 237 bp, Canis familiaris
atgacacatgcaagtgctcaataacgttagacactgtactgttaattaaaggtctatcgcccctttaaacaaaatgtccagaatgttcatgttcaccaaaagtgaaaggcattcatgtctmtgtttctgttgagttcactgtcacctttgtgcctagaaaggagaagacacactggtttttcctcctctagagaagtgcagatttgtataggtgaggagtatacataggttgtgggc

SEQ ID NO: 192 - DNA, 237 bp, Canis familiaris
ctttgggaatgaggcctgtcccgctagcctgcttcatttactctcatgattcttggcaaagttcttataagtcacgttcaaattatcaggcttcattcctagtctgagcagacttgtcccrtctcccagcctgtggatgttcaagaagcgcaacttggttttatgtttattaatcaaaagccctttagcctctgatgaacctctgagggtggctttaaagccccgcgcctgctctga

SEQ ID NO: 193 - DNA, 237 bp, Canis familiaris
aaagaaaaaagtaagggtcaaaacactagcaaaattaaattaaaaaaataagaaaaacaagtcacactttttttttttttttggtcatttgggaaaagcacaatattttgcttgattactyttcctcacttttcaactagtaatatagattgcatgaaaaataaacaaaacaagtaaactttaaatgtttgctggtgtagaggtgaataagaacaatccatggattttgcaatcaca

SEQ ID NO: 194 - DNA, 237 bp, Canis familiaris
tctagctccagtctcctttattcagtgccaccttcatttttccattccagccaaattagtgttttcattctctcaagcattttcatctatgtacttcctgaaccctcttcatggaagacaycctctactcttcagcatattactatcccagcatcccttaccctgatagtttaacttgattctttatctacctgattcagtaatatttctctattcttatcatattcagcaatgttc

SEQ ID NO: 195 - DNA, 237 bp, Canis familiaris
tcccctactgaaaacaaattcccccatcttcaccctaccatggggattttacatttgttaccagatttggggcaaactcatcctattttcccttcagtgtggagaagagattttggaaagyagaccatgcaaatctctaagctcacaataaactgaattggagaggcataaaacctgacaggaaaaaaaggtgtgaacttgatctttagcttgctgttctggtttaataggtttctg

SEQ ID NO: 196 - DNA, 237 bp, Canis familiaris
aagggtgaactgacttttagtcagaatgtttatttttaacagattataaaatagccacctatttagatggataaatgtattgtgattatggtgttgtttataaaaagaattttcaggattktccacaaaacttaatgttagtattagttattaagagtacaatggaatatcattcagccatataaaagaatgaaatcttgctatttgcaatgacatagatggagctagagagtataa

SEQ ID NO: 197 - DNA, 237 bp, Canis familiaris
atgagtttgcaattctagccggtgcatgaggacttctccctttcccgagccctcccggaaagtttggccagatccccagcccaaatggcagcatgtgctcgggaagatgattaatgttagygcgaggctccagagaatctctcagggcccttttgtttattaaatagaaaaattcatgtttaaatataatgtcaaggggatgacacggaccaacatgatccaagacagactgccggc

SEQ ID NO: 198 - DNA, 237 bp, Canis familiaris
ctcccactaactagcaggtatacatagttaaatttctctaacacagagcaatactaccttccacaccagaaaatggcaaaggctaaatataaccacagatctcaaggctactgaactacaygcaggtaatagattatatttaaaacatatcagatgaatctgcactaatactgggggcctataaaactttctaacatacagtagtataagcaggatttccaatcagtgagaaaagga

SEQ ID NO: 199 - DNA, 121 bp, Canis familiaris
atgtgtaatttacaaagagttcatatattactttatcagttaagcttttgtaattccatamtctatactaattttaaagaggagtgattccttcttgcaattagtttattgcctccgtatg

SEQ ID NO: 200 - DNA, 237 bp, Canis familiaris
atatatcattccacctatagtaattttcactaatctgcccatttattccctagtgcatacccttaatataaatctgcaacaagaatataacttttctaaaaaaaaaaaaaaagtgtacatrcattagtgatgtgtgtgaccaactaaataccagtgtataagcccatgcccatatttcattttcacgaattatgtttgctgcataaataagacttgtagctttttaaacttacctct

SEQ ID NO: 201 - DNA, 237 bp, Canis familiaris
gtgtcagtatgttaagccactagtgcactgttaactgctgccatgactaagaaaaaacacagaagctgctgctgctactatgtcactcttgtcatttttaaggtgaatcctcatatgaatragagggagtacatgcttaatggtcagagtgacagcttttgcttcatggcgagccatcgaaaccccacaaatctctttgccccaacagattcttcacctttcttctccagaaatgaa

SEQ ID NO: 202 - DNA, 237 bp, Canis familiaris
ttatggatcttacaatctagtgattgaaacacaaattagatttgggcttgtctataaaactgggatattttctgatattggaatgaatactgggacagtcccttaattatggtttcatgartgattagtcttatgatacatagtttatgtgtaattgctatttctaatccaaaataaattggacctttcgtttagattaaacatggagtctttgatgtaaataccgtagaaggagtc

SEQ ID NO: 203 - DNA, 237 bp, Canis familiaris
tgctgtctaaacaggagcttgaaggatgagtaggaagagatttcagatagaacagctgtgctggagcaaagagggtctgagggagcatggtatatttagtggacggcagctagttgcctgscactggagcatggcgggtggggagtaagaggtgggagagaaaactcaatgacaggcagaagccagaccatgaagggcctcacatcctgtgcagaggagttttgatttttatctcct

SEQ ID NO: 204 - DNA, 237 bp, Canis familiaris
tttgtccttgaaagaagtttttctctttctttcccattttctttttcttcctatttgcttaattatctgttgccagataattcacacctaagttcatagaggaccaatgtcacagatattytcttaaacaaaactggctttgtaacaataaaatttgtctgtttaaaatgtaactaatatcggagatatttacctaaggaagtatttgtaaatagtatctagaaatgcaagaaaata

SEQ ID NO: 205 - DNA, 237 bp, Canis familiaris
gccaacgctaagattcatatgtctatttttactcaacaccaaataaaggtaccatttctaatccaagaacttcactctgctgtcttctagcacattggcattttccacaggcatttcttgytttacttgatgtatttttttccagtttttcttaatatgatatctgagaaatttttttgctaagtattgattcaaaaatttaaaattaaggttaaattgtggctaatcagcatactg

SEQ ID NO: 206 - DNA, 236 bp, Canis familiaris
ttttatcatgccaggaaattcttggaatgtagccactgtctgatatttatggttccataagcatttgactctgaaaagtctctaattctggaaaacggccactgatcagttgttaatgcayagcagtaggaaaaaagtcaccccttaaaaggagagagaggacaaaaggaacagcttgtgaggctaaaagtatgacaagtatgacgtctacctatacaggaagtgtatatgcatct

SEQ ID NO: 207 - DNA, 121 bp, Canis familiaris
gctaataaaggatcaacctctgggctgcagaataacctaatctattcatacctcagtgacrtcctgaattagaaccgggggctgatgaactccaatgcaccagccaaccaaccagagttag

SEQ ID NO: 208 - DNA, 237 bp, Canis familiaris
tgaatgactttttcaacccgaattttcatgacatttttgtcatgacatttctcatataacctaccgcatgtaaagcaagatctcctattggattctgtcttattttttgtcatcttccaayggtcttaggcaaatgaagtttaagtagtaagattatatgcctcctcccactttggtgcatgcacacagatgcaggaacatgcttagtaactaatctttgtgggacataggaatgcc

SEQ ID NO: 209 - DNA, 237 bp, Canis familiaris
gccagctctaatgagtttgtttccaagcggtgcttccagaaattgttagtggttggtagttgcaatgggttttgaaattagaggacatcacagcagagtagaatggtttggaacaggggartatgattaggattaatgagatgaaagaaaattctggctagagggctagaagagccatggaagaaaatatacactaaccctttggagtgttcctccaagtgaagatttgcaacattt

SEQ ID NO: 210 - DNA, 237 bp, Canis familiaris
acgagaagcaagattgccataccgttcctggtaccgggccatgacgttgaccttcaaaagccctgaaacggctgttttcctggctgctgtgagctgtggaactcaggagtaggtatttccygaaaacatttaacatcccatagcaaaggtgttggaggcgtcgtctccattgtcgtttctcccgggctgtggttggcctttctgcgtgagtgcttctccccgctgcgggctggctct

SEQ ID NO: 211 - DNA, 237 bp, Canis familiaris
taggaaaaaacatctggcctctgactcggatccagtcatcccagcctcattcacacccacccatcagctctcagagaaccttctgagacttcgataaatagctgagcccttaaaatgacarcattgatttggcatggtttgggcaataacttctggctgctgtgatttttaggttttgaatatttagtttctggaaactctgatagaatgaataactttatatgtttatttaattct

SEQ ID NO: 212 - DNA, 237 bp, Canis familiaris
gtctactgaagccagacagttggttcattagattaattaaagtgcaaactaaccccaatctggtgttttgataacggccacagggctcttgaagttggaatcggccagcatttgacagtgytctcattaaagccacagtggaattgcctctatggtttctcctaaacttttgaatttaccttataacaaagaagtggactttgagcatccctgattgttttttcagtgttaactgct

SEQ ID NO: 213 - DNA, 237 bp, Canis familiaris
tgttgctttcctgcacacaagcagttgaaccagagtagggaggaatcatttttaggaatgtgttattattattttttaggaatgcacaaaacccatgccaaaaagcccatccacgtctaaygtccttgaacctctccttcactaccaattgtattcttttatgttcccaatcaactggctggcctgaaatagatttctcctaccaagaaatgtagataaaaatatttatttctggaa

SEQ ID NO: 214 - DNA, 237 bp, Canis familiaris
gtctcagccctctattccagaaggtaggactggccctgggcctgtctacgaggtggtggctgcgagccctcaaggcctggcattgtcaaagttctgacaaccttccccacctatggcagckcagtgttagacgctccaggctgagggttgatgcacactttttcggcttccaaagtgtggccttctcctcagggcttcccatggggtccacaggctggcagcaacctcttggagaaa

SEQ ID NO: 215 - DNA, 237 bp, Canis familiaris
cagctgtgtcatggaaatggcactttaaaaattcatatgaatcttaacagtaaagcacaagactttggagatatttctcctgttgaatagctgcttggggatgtgccacagatctgtagargtcagcattcactctaagttcccgggaaccatgagacagcagcaaccatggccaccacagcaacacagcaggtgcccataagcccattttacagatggagaaattgggtccagaga

SEQ ID NO: 216 - DNA, 237 bp, Canis familiaris
cctctggctccccagaacctcagagcttaggggatgtagtggttgtaatcctggatccctctgtggggtggcaggtctggagtggtgagctactgtgagggaactggggtaactgtgaccygagaagaaaggagcgagggagtgagtgtgtgtctgtgaaatatgcctctgtgtgtataaacagggctggagggctcagtgccccccactcccaaagatccacctgttacatccccg

SEQ ID NO: 217 - DNA, 237 bp, Canis familiaris
ttcttctcttgtgactggtcactaaagacagagatttcaggagagctgactttggtaggaattctcacccttttctggcctaggcctataatttttataccgacagctggagtcccagatrgaagagaccttaaactctttggactatgaagaacctgttttttctctctctctcttttttttccccttaaaacaaaaatttattttcctcaggcctcatcctgtacccagtcttgt

SEQ ID NO: 218 - DNA, 237 bp, Canis familiaris
agctccaatttagtcatatactaaagaatcaggtcatactctaggcagactctaggcagttagcacatgaaaccagttcacatgctttatcatcatcctttttgttctcaaaacagccaamaacagttctgtataagatatttcacatgtttaattctttcagttcttctagcaagcaggaagcttagaacaagattttagtatttggtttagataacaattgcaaataggagcacc

SEQ ID NO: 219 - DNA, 237 bp, Canis familiaris
gacttttctagagagaccatggaagatgcatgtggggcctgcccaggctgccacaggggaaaggagccgggaggagggagctgtcaggccacttcctctgatggcccctcagcagcaggargagagcatttcctcaccagatcccactcaacactggccacggtccccctgtggacttcagaactgactcagaactaacctgactgactgcgtatgatttgtctttttaggaggacc

SEQ ID NO: 220 - DNA, 237 bp, Canis familiaris
cccgcgccaggccggtcctctcctcccagctcctcctctcccgctcgcagtcagggcagccagggaggggagaaattctcatctcaaaactagtaagacaaggccccgcagcgggtctgcrgcgcggaggcggctgcctctcctggtccatactggacacagctgaccacatttcaacaggtaagaatcattttaaatattacccttaaaccaaaaaaagttcttcttttgcttcta

SEQ ID NO: 221 - DNA, 237 bp, Canis familiaris
cagtattccgattcttctatttgctaattttaaagtgcagatctaagaggacaaccttattattatttccatggtcttagagatcatcttactgttgccccacaatgtccatgcttcccgkgaaagatgtgtgtatccagactcaaagtgaatctaatagggaaggaagactgagaattctattagtaagcaacccgtatttaacaacatggcccagtttgaagatttgcagaaaca

SEQ ID NO: 222 - DNA, 237 bp, Canis familiaris
tcaggagtgagcctgtacgttatcctgactactgattcccttgcaccaaaaaagcaacgggagcataagggcaagatatgacctttagctaaagggttgcaagttatattactagtcgtcrctgctcaaacacccagcaccagaccctgcatagaatacagaaaagagtcctcaccatcaagccactaccacctgaagcatgaaggagagaacaaggagagatcacctcctaagtgt

SEQ ID NO: 223 - DNA, 237 bp, Canis familiaris
ctgacctctgctctagtcaattgctctgaaagtacagtcctctgatcctagactcgaaccctctcaagcataacagttccatctactattcactaatccatttatttaactgggagtgttstatgctttggctctgggatatgaaggaaaggacattgtgcccgaacatataggaaagttattgtttaaggagatatacagggaaataattttaaaacaccatggtaatcttttcct

SEQ ID NO: 224 - DNA, 237 bp, Canis familiaris
cgttttccttataaatttttagaaaacagaacaggaaaaaaaaaaaaagaaagaaaacagaacagagaacaaaccaacatgtcttgatgcctccaggaaccagttttctcatagccttagrggaaacaatttacaaaatatctgaaaagcctgcagatatcttagatccaagattccaaggcataaaaatgtaagtgatcatgtactacgtattactgaaatacagaaagcaaccaa

SEQ ID NO: 225 - DNA, 237 bp, Canis familiaris
agcaccttgagaatggtgtagtggaaagaaagttgacttttagtaactatgcatttgtctcgttaatgcagtttctcacctgctttgagataatgggaaatggaactaacaggtagtggtracacagatgatggacaatataaagatttgagatatatataaaaaaaatttgatcattatatgtacactttgctagttttgctctacattttttatccacacaaaaagtaatttgca

SEQ ID NO: 226 - DNA, 237 bp, Canis familiaris
taagtagcctttagtgcaaggaaaagaaaaaggcagtaaggatgaacctttgtttcaaaggtattaggagtcatttaaggaatttcaaaaaaaaaaaaaagaagtgacatgattttgaacraagaagtgactgtcagtactataaagagcacattgcctcaaggagaaactgaagttagagaagccaaattggctgataaaaatctaggccggagatgcaaacacctaaatgaaaac

SEQ ID NO: 227 - DNA, 20 bp, Artificial Sequence
  Primer
gttaccctgcagctgagagt

SEQ ID NO: 228 - DNA, 20 bp, Artificial Sequence
  Primer
atggcgagcatcacagtatc

SEQ ID NO: 229 - DNA, 37 bp, Artificial Sequence
  Primer
gttttcccagtcacgacgttaccctgcagctgagagt

SEQ ID NO: 230 - DNA, 17 bp, Artificial Sequence
  Primer
gttttcccagtcacgac

SEQ ID NO: 231 - DNA, 19 bp, Artificial Sequence
  Primer
gttaccctgcagctgagag

SEQ ID NO: 232 - DNA, 20 bp, Artificial Sequence
  Primer
agggtcgtactgtacttggg

SEQ ID NO: 233 - DNA, 21 bp, Artificial Sequence
  Primer
cgtctggatgggaagtttctc

SEQ ID NO: 234 - DNA, 19 bp, Artificial Sequence
  Primer
ttgtcggacttcagggagg

SEQ ID NO: 235 - DNA, 20 bp, Artificial Sequence
  Primer
ccggcggtgggactccccgc

SEQ ID NO: 236 - DNA, 989 bp, Canis familiaris
tcagcacccaggaggcagtcatcacttaccagccttatcttattcaaccccaggacctcagggaccatgtaaacgacatggggtttgaagctgtcatcaagaacagagtggcacccgtaagcctgggacccattgatattgggcggttacagaggaccaacccaaagatgcctttgacttctgataaccagaatctcaataactctgagaccttgggccatcaagggagccatgtggttaccctgcagctgagagtcgacggaatgcactgtcagtcttgtgtcctgaacattgaagagaatataggccaactccccggggttcagaatgtgcaagtgtccttggagaacagaacggcccaagtacagtacgacccttcttgtgtcaccgcaggggccctgcagagggccattgaagctctcccaccagggaactttaaagtttctcttcctgccgcagcagcaggaagtgagacaggtaacaggttttcggcatgtgccgcccccgccccaagaaccccggcaccgggcaggtgcgatactgtgatgctcgccattgtgggcatgacctgtgcatcctgcgtccagtcgatcgaaggcctgatctcccagagggaaggggtgcagcaaatatctgtctctctggctgaagggaccgcagtggttctctatgatccctctataattggcccggaagaactccgagctgccgtcgaggagatgggatttgagacttcagtcctctctggtatgtagtggcaccccgggtcttctcctctctccttgggccttacggcagagtgcctgcagggtggcacaggggagccaccccagctgctcgcctgtcgggttggccaagtcccgcagcgtttccctgtgtgttgaatgtgtccgggtgggagaaagagaactttctggtgtgtagattttgcctctcatggggctgggactacattgctaaattctttgttgttgttattttttttaact

SEQ ID NO: 237 - DNA, 995 bp, Canis familiaris
tcagcacccaggaggcagtcatcacttaccagccttatcttattcaaccccaggacctcagggaccatgtaaacgacatggggtttgaagctgtcatcaagaacagagtggcacccgtaagcctgggacccattgatattgggcggttacagaggaccaacccaaagatgcctttgacttctgataaccagaatctcaataactctgagaccttgggccatcaagggagccatgtggttaccctgcagctgagagtcgacggaatgcactgtcagtcttgtgtcctgaacattgaagagaatataggccaactccccggggttcagaatgtgcaagtgtccttggagaacagaacggcccaagtacagtacgacccttcttgtgtcaccgcaggggccctgcagagggccattgaagctctcccaccagggaactttaaagtttctcttcctgccgcagcagcaggaagtgagacaggtaacaggttttcggcatgtgccgcccccgcccccgccccaagaaccccggcaccgggcaggtgcgatactgtgatgctcgccattgtgggcatgacctgtgcatcctgcgtccagtcgatcgaaggcctgatctcccagagggaaggggtgcagcaaatatctgtctctctggctgaagggaccgcagtggttctctatgatccctctataattggcccggaagaactccgagctgccgtcgaggagatgggatttgagacttcagtcctctctggtatgtagtggcaccccgggtcttctcctctctccttgggccttacggcagagtgcctgcagggtggcacaggggagccaccccagctgctcgcctgtcgggttggccaagtcccgcagcgtttccctgtgtgttgaatgtgtccgggtgggagaaagagaactttctggtgtgtagattttgcctctcatggggctgggactacattgctaaattctttgttgttgttattttttttaact

SEQ ID NO: 238 - DNA, 1001 bp, Canis familiaris
tcagcacccaggaggcagtcatcacttaccagccttatcttattcaaccccaggacctcagggaccatgtaaacgacatggggtttgaagctgtcatcaagaacagagtggcacccgtaagcctgggacccattgatattgggcggttacagaggaccaacccaaagatgcctttgacttctgataaccagaatctcaataactctgagaccttgggccatcaagggagccatgtggttaccctgcagctgagagtcgacggaatgcactgtcagtcttgtgtcctgaacattgaagagaatataggccaactccccggggttcagaatgtgcaagtgtccttggagaacagaacggcccaagtacagtacgacccttcttgtgtcaccgcaggggccctgcagagggccattgaagctctcccaccagggaactttaaagtttctcttcctgccgcagcagcaggaagtgagacaggtaacaggttttcggcatgtgccgcccccgcccccgcccccgccccaagaaccccggcaccgggcaggtgcgatactgtgatgctcgccattgtgggcatgacctgtgcatcctgcgtccagtcgatcgaaggcctgatctcccagagggaaggggtgcagcaaatatctgtctctctggctgaagggaccgcagtggttctctatgatccctctataattggcccggaagaactccgagctgccgtcgaggagatgggatttgagacttcagtcctctctggtatgtagtggcaccccgggtcttctcctctctccttgggccttacggcagagtgcctgcagggtggcacaggggagccaccccagctgctcgcctgtcgggttggccaagtcccgcagcgtttccctgtgtgttgaatgtgtccgggtgggagaaagagaactttctggtgtgtagattttgcctctcatggggctgggactacattgctaaattctttgttgttgttattttttttaact